European Patent Specification EP 3 887 525 B1, published August 23, 2023. Title: COMPOSITION FOR PREVENTING OR TREATING PULMONARY DISEASES COMPRISING HYALURONAN AND PROTEOGLYCAN LINK PROTEIN 1. Applicant: HAPLNSCIENCE INC. The sequence listing filed with the application follows.

SEQUENCE LISTING (1 sequence)

SEQ ID NO: 1 - protein, 339 aa, Artificial Sequence
  Recombinant human HAPLN1
DHLSDNYTLDHDRAIHIQAENGPHLLVEAEQAKVFSHRGGNVTLPCKFYRDPTAFGSGIHKIRIKWTKLTSDYLKEVDVFVSMGYHKKTYGGYQGRVFLKGGSDSDASLVITDLTLEDYGRYKCEVIEGLEDDTVVVALDLQGVVFPYFPRLGRYNLNFHEAQQACLDQDAVIASFDQLYDAWRGGLDWCNAGWLSDGSVQYPITKPREPCGGQNTVPGVRNYGFWDKDKSRYDVFCFTSNFNGRFYYLIHPTKLTYDEAVQACLNDGAQIAKVGQIFAAWKILGYDRCDAGWLADGSVRYPISRPRRRCSPTEAAVRFVGFPDKKHKLYGVYCFRAYN